European Patent Application EP 4 269 612 A1, published November 1, 2023. Title: NUCLEIC ACID AMPLIFICATION METHOD, PRIMER SET, PROBE, AND KIT FOR NUCLEIC ACID AMPLIFICATION METHOD. Applicant: EIKEN KAGAKU KABUSHIKI KAISHA. The sequence listing filed with the application follows.

SEQUENCE LISTING (24 sequences)

SEQ ID NO: 1 - DNA, 92 bp, Artificial Sequence
  miR-21-5p Fw adapter nucleotide
taacgagcggcttccccaaaccgtctttcaccacatcgcattatatcgttcttctaaatcaaagtaggaagccgctcgttatagcttatcag

SEQ ID NO: 2 - DNA, 98 bp, Artificial Sequence
  miR-21-5p Bw adapter primer CT
gcaactcaatccgttgaaaagagcggtatccccatcatcatcgacaaggtttataatttgggcagcgacatcaacggattgagttgctcaacatcagt

SEQ ID NO: 3 - RNA, 22 nt, Homo sapiens
uagcuuaucagacugauguuga

SEQ ID NO: 4 - DNA, 92 bp, Artificial Sequence
  Let-7a-5p Fw adapter nucleotide
taacgagcggcttccccaaaccgtctttcaccacatcgcattatatcgttcttctaaatcaaagtaggaagccgctcgttatgaggtagtag

SEQ ID NO: 5 - DNA, 98 bp, Artificial Sequence
  Let-7a-5p Bw adapter primer CT
gcaactcaatccgttgaaaagagcggtatccccatcatcatcgacaaggtttataatttgggcagcgacatcaacggattgagttgcaactatacaac

SEQ ID NO: 6 - RNA, 22 nt, Homo sapiens
ugagguaguagguuguauaguu

SEQ ID NO: 7 - DNA, 98 bp, Artificial Sequence
  miR-21-5p Bw adapter primer ST1
tcaacggattgagttgcaaagagcggtatccccatcatcatcgacaaggtttataatttgggcagcgacatcaacggattgagttgctcaacatcagt

SEQ ID NO: 8 - DNA, 98 bp, Artificial Sequence
  miR-21-5p Bw adapter primer ST2
catcatcgacaaggtttaaagagcggtatccccatcatcatcgacaaggtttataatttgggcagcgacatcaacggattgagttgctcaacatcagt

SEQ ID NO: 9 - DNA, 81 bp, Artificial Sequence
  Let-7a-5p Bw adapter primer D1
aaagagcggtatccccatcatcatcgacaaggtttataatttgggcagcgacatcaacggattgagttgcaactatacaac

SEQ ID NO: 10 - DNA, 98 bp, Artificial Sequence
  Let-7a-5p Bw adapter primer ST1
tcaacggattgagttgcaaagagcggtatccccatcatcatcgacaaggtttataatttgggcagcgacatcaacggattgagttgcaactatacaac

SEQ ID NO: 11 - DNA, 98 bp, Artificial Sequence
  Let-7a-5p Bw adapter primer ST2
catcatcgacaaggtttaaagagcggtatccccatcatcatcgacaaggtttataatttgggcagcgacatcaacggattgagttgcaactatacaac

SEQ ID NO: 12 - DNA, 19 bp, Artificial Sequence
  PCR-F-primer
ccaaaccgtctttcaccac

SEQ ID NO: 13 - DNA, 18 bp, Artificial Sequence
  PCR-B-primer
aaagagcggtatccccat

SEQ ID NO: 14 - DNA, 19 bp, Artificial Sequence
  Fw inner primer
ccaaaccgtctttcaccac

SEQ ID NO: 15 - DNA, 18 bp, Artificial Sequence
  Bw inner primer
aaagagcggtatccccat

SEQ ID NO: 16 - DNA, 11 bp, Artificial Sequence
  Probe designed in miR-21-5p region
cagtctgataa

SEQ ID NO: 17 - DNA, 11 bp, Artificial Sequence
  Probe designed in Let-7a-5p region
caacctactac

SEQ ID NO: 18 - DNA, 28 bp, Artificial Sequence
  Probe designed in loop region
  misc_feature (26)..(26): n is inosine
cgacaaggtttataatttgggcagcnac

SEQ ID NO: 19 - DNA, 10 bp, Artificial Sequence
  miRNA21Probe-2
cttatcagac

SEQ ID NO: 20 - DNA, 11 bp, Artificial Sequence
  miRNA21Probe-3
cttatcagact

SEQ ID NO: 21 - DNA, 13 bp, Artificial Sequence
  miRNA21Probe-4
cttatcagactga

SEQ ID NO: 22 - DNA, 16 bp, Artificial Sequence
  miRNA21Probe-5
cttatcagactgatgt

SEQ ID NO: 23 - DNA, 19 bp, Artificial Sequence
  miRNA21Probe-6
cttatcagactgatgttga

SEQ ID NO: 24 - DNA, 10 bp, Artificial Sequence
  miRNA21Probe-7
caacatcagt